European Patent Application EP 4 454 665 A1, published October 30, 2024. Title: Composition for preventing and treating ischemia-reperfusion injury and use thereof. Applicant: NA Vaccine Institute. The sequence listing filed with the application follows.

SEQUENCE LISTING (6 sequences)

SEQ ID NO: 1 - RNA, 429 nt, synthetic construct
  source 1..429: mol_type = other RNA
gggcgataatacagttttggactcaggtgtgagattttatgatcaggactatgaaggacaaataaccccaatggaatatgtaactgggttgtataacttttggtcagggccaatagagttacgttttgattttgtttcaaatgcgtttcacactggaacagtgattatatcagcggagtataatcgatcatctactaatacggatgagtgtcagtcacactcaacttatactaaaacgttccacttgggagaacaaaaatcagtacatttcactgtgccttatatatatgatactgttatgcggagaaatacggctagcgcctatttaccggtaactgattatgataaggcagataatgttagtagggcgcaggctacggggattagagcagaatctaaaatgagagtgaaagtgagatcgccctatag

SEQ ID NO: 2 - RNA, 429 nt, synthetic construct
  source 1..429: mol_type = other RNA
gggcgatctcactttcactctcattttagattctgctctaatccccgtagcctgcgccctactaacattatctgccttatcataatcagttaccggtaaataggcgctagccgtatttctccgcataacagtatcatatatataaggcacagtgaaatgtactgatttttgttctcccaagtggaacgttttagtataagttgagtgtgactgacactcatccgtattagtagatgatcgattatactccgctgatataatcactgttccagtgtgaaacgcatttgaaacaaaatcaaaacgtaactctattggccctgaccaaaagttatacaacccagttacatattccattggggttatttgtccttcatagtcctgatcataaaatctcacacctgagtccaaaactgtattatcgccctatag

SEQ ID NO: 3 - DNA, 18 bp, synthetic construct
  source 1..18: mol_type = other DNA
taatacgactcactatag

SEQ ID NO: 4 - DNA, 533 bp, synthetic construct
  source 1..533: mol_type = other DNA
cggtacctcgcgaatgcatctagatatcggatcctaatacgactcactatagggcgataatacagttttggactcaggtgtgagattttatgatcaggactatgaaggacaaataaccccaatggaatatgtaactgggttgtataacttttggtcagggccaatagagttacgttttgattttgtttcaaatgcgtttcacactggaacagtgattatatcagcggagtataatcgatcatctactaatacggatgagtgtcagtcacactcaacttatactaaaacgttccacttgggagaacaaaaatcagtacatttcactgtgccttatatatatgatactgttatgcggagaaatacggctagcgcctatttaccggtaactgattatgataaggcagataatgttagtagggcgcaggctacggggattagagcagaatctaaaatgagagtgaaagtgagatcgccctatagtgagtcgtattagtcgactgcagaggcctgcatgcaagcttggcgtaatcatg

SEQ ID NO: 5 - DNA, 18 bp, synthetic construct
  source 1..18: mol_type = other DNA
cggtacctcgcgaatgca

SEQ ID NO: 6 - DNA, 20 bp, synthetic construct
  source 1..20: mol_type = other DNA
catgattacgccaagcttgc